European Patent Specification EP 4 395 806 B1, published October 22, 2025. Title: PROTEIN COMPOSITIONS FOR THE TREATMENT OF INFLAMMATORY DISEASES. Applicant: UNICHEM LABORATORIES LIMITED. The sequence listing filed with the application follows.

SEQUENCE LISTING (4 sequences)

SEQ ID NO: 1 - protein, 141 aa, Sclerotium rolfsii
TYKITVRVYQTNPNAFFHPVEKTVWKYANGGTWTITDDQHVLTMGGSGTSGTLRFHADNGESFTATFGVHNYKRWCDIVTNLAADETGMVINQQYYSQKNREEARERQLSNYEVKNAKGRNFEIVYTEAEGNDLHANLIIG

SEQ ID NO: 2 - protein, 141 aa, synthetic construct
TYKITVRVYQTNPDAFFHPVEKTVWKYANGGTWTITDDQHVLTMGGSGTSGTLRFHADNGESFTATFGVHNYKRWCDIVTNLAADETGMVINQQYYSQKNREEARERQLSNYQVKNAKGRNFQIVYTEAEGNDLHANLIIG

SEQ ID NO: 3 - protein, 141 aa, synthetic construct
VYKITVRVYQTNPDAFFHPVEKTVWKYANGGTWSITDDQHVLTMGGSGTSGTLRFHADNGESFTATFGVHNYKRWCDIVTNLAADETGMVINQQYYSQKNREEARERQLSNYQVKNAKGRNFQIVYTEAEGNDLHANLIIG

SEQ ID NO: 4 - protein, 141 aa, synthetic construct
VYKITVRVYQTNPDAFFHPVEKTVWKYADGGTWSITDDQHVLTMGGSGTSGTLRFHADNGESFTATFGVHDYKRWCDIVTDLAADETGMVINQEYYSEKDREEARERQNSNYEVKDAKGRNFEIVYTEAEGNDLHADLIIG